European Patent Specification EP 3 546 481 B1, published November 8, 2023. Title: Anti-interleukin 22 (IL-22) antibody and uses thereof. Applicant: ImmunoQure AG. The sequence listing filed with the application follows.

SEQUENCE LISTING (81 sequences)

SEQ ID NO: 1 - DNA, 20 bp, Artificial Sequence
  Oligonucleotide (primer) 6F
tgcaggctgtgggaactcca

SEQ ID NO: 2 - DNA, 22 bp, Artificial Sequence
  Oligonucleotide (primer) 6R
agaaaaagagctgtaccctgtg

SEQ ID NO: 3 - DNA, 22 bp, Artificial Sequence
  Oligonucleotide (primer) 3R
tgcaaggaagaggggcgtcagc

SEQ ID NO: 4 - DNA, 21 bp, Artificial Sequence
  Oligonucleotide (primer) 49300F
tccaccacaagccgaggagat

SEQ ID NO: 5 - DNA, 21 bp, Artificial Sequence
  Oligonucleotide (primer) 49622R
acgggctcctcaaacaccact

SEQ ID NO: 6 - DNA, 378 bp, Homo sapiens
  CDS (1)..(378): 9A2-VH variable heavy chain (VH) sequence; 9A2: IgG1, kappa
  V_region (91)..(105): complementarity determining region (CDR) VH-CDR1
  V_region (148)..(198): complementarity determining region (CDR) VH-CDR2
  V_region (295)..(345): complementarity determining region (CDR) VH-CDR3
gaggtgcaattggaggagtctggcggaggcttggttcagcctggagggtccctgagactctcctgtgcagcctctggattccccttcagcaactatgaaatgaattgggtccgccaggctcccgggaagggactggagtggatttcatacattagtgtgagcggtggtcccgctcactacgcagactctgtgaagggccgattcaccatttccagagacgacgccacaaagtcactgtttctgcaaatgaaccgcctgagagccgacgacacggcagtttattactgtgtgcgccgcgaatatgtcactggccgcaattacaactactacccctacatggacgtctggggcactgggaccacggtcaccgtctcccca

SEQ ID NO: 7 - protein, 126 aa, Homo sapiens
EVQLEESGGGLVQPGGSLRLSCAASGFPFSNYEMNWVRQAPGKGLEWISYISVSGGPAHYADSVKGRFTISRDDATKSLFLQMNRLRADDTAVYYCVRREYVTGRNYNYYPYMDVWGTGTTVTVSP

SEQ ID NO: 8 - DNA, 321 bp, Homo sapiens
  CDS (1)..(321): 9A2-VL variable light chain (VL) sequence, kappa type
  V_region (70)..(102): complementarity determining region (CDR) VL-CDR1
  V_region (148)..(168): complementarity determining region (CDR) VL-CDR2
  V_region (265)..(291): complementarity determining region (CDR) VL-CDR3
gacatccagatgacccagtctccgtcctccctgtctgcttctgttggggacagagtcaccatcacttgccgggcaagtcagaccataagtgattatttaaattggtaccagcacaaaccaggggaagcccctaaactcctaatctattctgcatccaccttgcaacgtggggtgccttcacggttcagtggcagtggatctgggacagatttcgttttcaccattagtagtctgcagtctgatgattttgcgacttactactgtcaacagacttccagtaccgccctcactttcggcggagggaccaaggtggaggtcaaa

SEQ ID NO: 9 - protein, 107 aa, Homo sapiens
DIQMTQSPSSLSASVGDRVTITCRASQTISDYLNWYQHKPGEAPKLLIYSASTLQRGVPSRFSGSGSGTDFVFTISSLQSDDFATYYCQQTSSTALTFGGGTKVEVK

SEQ ID NO: 10 - DNA, 993 bp, Homo sapiens
  CDS (1)..(990): 9A2-CH constant heavy chain (CH) sequence
gcctccaccaagggcccatcggtcttccccctggcaccctcctccaagagcacctctgggggcacagcggccctgggctgcctggtcaaggactacttccccgaaccggtgacggtgtcgtggaactcaggcgccctgaccagcggcgtgcacaccttcccggctgtcctacagtcctcaggactctactccctcagcagcgtggtgaccgtgccctccagcagcttgggcacccagacctacatctgcaacgtgaatcacaagcccagcaacaccaaggtggacaagaaagttgagcccaaatcttgtgacaaaactcacacatgcccaccgtgcccagcacctgaactcctggggggaccgtcagtcttcctcttccccccaaaacccaaggacaccctcatgatctcccggacccctgaggtcacatgcgtggtggtggacgtgagccacgaagaccctgaggtcaagttcaactggtacgtggacggcgtggaggtgcataatgccaagacaaagccgcgggaggagcagtacaacagcacgtaccgtgtggtcagcgtcctcaccgtcctgcaccaggactggctgaatggcaaggagtacaagtgcaaggtctccaacaaagccctcccagcccccatcgagaaaaccatctccaaagccaaagggcagccccgagaaccacaggtgtacaccctgcccccatcccgggatgagctgaccaagaaccaggtcagcctgacctgcctggtcaaaggcttctatcccagcgacatcgccgtggagtgggagagcaatgggcagccggagaacaactacaagaccacgcctcccgtgctggactccgacggctccttcttcctctacagcaagctcaccgtggacaagagcaggtggcagcaggggaacgtcttctcatgctccgtgatgcatgaggctctgcacaaccactacacgcagaagagcctctccctgtctccgggtaaatga

SEQ ID NO: 11 - protein, 330 aa, Homo sapiens [sequence omitted]

SEQ ID NO: 12 - DNA, 324 bp, Homo sapiens
  CDS (1)..(321): 9A2-CL constant kappa chain (CL) sequence
  misc_feature (260)..(260): not sequenced but obtained from database
  misc_feature (298)..(324): not sequenced but obtained from database
cgaactgtggctgcaccatctgtcttcatcttcccgccatctgatgagcagttgaaatctggaactgcctctgttgtgtgcctgctgaataacttctatcccagagaggccaaagtacagtggaaggtggataacgccctccaatcgggtaactcccaggagagtgtcacagagcaggacagcaaggacagcacctacagcctcagcagcaccctgacgctgagcaaagcagactacgagaaacacaaagtctacgcctgcgaagtcacccatcagggcctgagctcgcccgtcacaaagagcttcaacaggggagagtgttag

SEQ ID NO: 13 - protein, 107 aa, Homo sapiens [sequence omitted]

SEQ ID NO: 14 - DNA, 387 bp, Homo sapiens
  CDS (1)..(387): 17E3-VH variable heavy chain (VH) sequence; 17E3: IgG1, kappa
  V_region (91)..(105): complementarity determining region (CDR) VH-CDR1
  V_region (148)..(198): complementarity determining region (CDR) VH-CDR2
  V_region (295)..(354): complementarity determining region (CDR) VH-CDR3
caggtgcaactggtccagtctggggctgaagtggcgaagcctggggcctcagtgagactttcctgcaaggcgtctggattcagttttatcaagtattatatgcactgggtgcgacaggcccctggacaagggcttgagtggatgggggtcatcgagcccaccggtggtggcacaagctccgcacagaagttccgagacagagtcaccctgagcagggacacgtccacggccactgtccatttggaagtgagtaggctgactcttgaggacacgggcatttatttctgtgtgagagactccatatattgtaaacatgggacctgtcatcggactgtgatcgatgcttttgacatttggggccaagggacggcggtcaccgtctcttca

SEQ ID NO: 15 - protein, 129 aa, Homo sapiens
QVQLVQSGAEVAKPGASVRLSCKASGFSFIKYYMHWVRQAPGQGLEWMGVIEPTGGGTSSAQKFRDRVTLSRDTSTATVHLEVSRLTLEDTGIYFCVRDSIYCKHGTCHRTVIDAFDIWGQGTAVTVSS

SEQ ID NO: 16 - DNA, 324 bp, Homo sapiens
  CDS (1)..(324): 17E3-VL variable light chain (VL) sequence, kappa type
  V_region (70)..(102): complementarity determining region (CDR) VL-CDR1
  V_region (148)..(168): complementarity determining region (CDR) VL-CDR2
  V_region (265)..(294): complementarity determining region (CDR) VL-CDR3
gacatccagatgacccagtctccatcctccctgtctgcatcagtaggagaccgagtcaccatcacttgccggtcaagtcaggacataaaaaatgatttagcctggtatcagcagaagccaggaaaagcccctgagcgcctgatctatgctgcatccaatttgcagagtggggtcccatcaaggttcagcggcagtggctctgggacagaattcagtcttacaatcagtggcctgcagcctgaagattttgcaacttattactgtctacagcataatagttaccctctgctcactttcggcggagggaccaaggtggagatcaaa

SEQ ID NO: 17 - protein, 108 aa, Homo sapiens
DIQMTQSPSSLSASVGDRVTITCRSSQDIKNDLAWYQQKPGKAPERLIYAASNLQSGVPSRFSGSGSGTEFSLTISGLQPEDFATYYCLQHNSYPLLTFGGGTKVEIK

SEQ ID NO: 18 - DNA, 993 bp, Homo sapiens; identical to SEQ ID NO: 10
  CDS (1)..(990): 17E3-CH constant heavy chain (CH) sequence

SEQ ID NO: 19 - protein, 330 aa, Homo sapiens [sequence omitted]

SEQ ID NO: 20 - DNA, 324 bp, Homo sapiens; identical to SEQ ID NO: 12
  CDS (1)..(321): 17E3-CL constant kappa chain (CL) sequence
  misc_feature (298)..(324): not sequenced but obtained from database

SEQ ID NO: 21 - protein, 107 aa, Homo sapiens [sequence omitted]

SEQ ID NO: 22 - DNA, 372 bp, Homo sapiens
  CDS (1)..(372): 24D3-VH variable heavy chain (VH) sequence; 24D3: IgG1, lambda
  V_region (91)..(105): complementarity determining region (CDR) VH-CDR1
  V_region (148)..(204): complementarity determining region (CDR) VH-CDR2
  V_region (301)..(339): complementarity determining region (CDR) VH-CDR3
gaggtgaagttggaggagtctgggggagacctggtaaagcctggggggtctcttagactctcctgtgtagcctctggattcactttcggcaccgcctggatgagctgggtccgccaggctccagggaaggggctggagtgggttggccgtattagcaacaaagacactggtgggagaatagactacgccgcacccgtgagaggcagattcgccatctcaagagatgattcgaaagccaccctgtttctgcaaatgaacagcctgaaaaccgaggacacagccgtgtatttttgtactacaaatttttacgatgttttgactggtgatcatgttgactattggggccagggaaccgtggtcgtcgtctcctca

SEQ ID NO: 23 - protein, 124 aa, Homo sapiens
EVKLEESGGDLVKPGGSLRLSCVASGFTFGTAWMSWVRQAPGKGLEWVGRISNKDTGGRIDYAAPVRGRFAISRDDSKATLFLQMNSLKTEDTAVYFCTTNFYDVLTGDHVDYWGQGTVVVVSS

SEQ ID NO: 24 - DNA, 318 bp, Homo sapiens
  CDS (1)..(318): 24D3-VL variable light chain (VL) sequence, lambda type
  V_region (67)..(99): complementarity determining region (CDR) VL-CDR1
  V_region (145)..(165): complementarity determining region (CDR) VL-CDR2
  V_region (262)..(288): complementarity determining region (CDR) VL-CDR2
tcctatgagctgacacagccaccctcggtgtcagtgtccccaggagagacggccaggatcccctgctctggagaaacattgccaaagaaacttgtttattggtatcagcagaagccaggccaggcccctgtattgatgatttataaagacagtgagaggccctcacgaatatctgagcgattctctggctccaactcagggacaatggcctccttgaccatcagtggagtccaggcagaagacgaggctgactattactgtcaaacatcagacagcagtggtgtggttttcggcggagggaccaagttgaccgtctta

SEQ ID NO: 25 - protein, 106 aa, Homo sapiens
SYELTQPPSVSVSPGETARIPCSGETLPKKLVYWYQQKPGQAPVLMIYKDSERPSRISERFSGSNSGTMASLTISGVQAEDEADYYCQTSDSSGVVFGGGTKLTVL

SEQ ID NO: 26 - DNA, 993 bp, Homo sapiens; identical to SEQ ID NO: 10
  CDS (1)..(990): 24D3-CH constant heavy chain (CH) sequence

SEQ ID NO: 27 - protein, 330 aa, Homo sapiens [sequence omitted]

SEQ ID NO: 28 - DNA, 321 bp, Homo sapiens
  CDS (1)..(318): 24D3-CL constant lambda chain (CL) sequence
  misc_feature (250)..(321): not sequenced but obtained from database
ggtcagcccaaggctgccccctcggtcactctgttcccgccctcctctgaggagcttcaagccaacaaggccacactggtgtgtctcataagtgacttctacccgggagccgtgacagtggcctggaaggcagatagcagccccgtcaaggcgggagtggagaccaccacaccctccaaacaaagcaacaacaagtacgcggccagcagctatctgagcctgacgcctgagcagtggaagtcccacagaagctacagctgccaggtcacgcatgaagggagcaccgtggagaagacagtggcccctacagaatgttcatag

SEQ ID NO: 29 - protein, 106 aa, Homo sapiens
GQPKAAPSVTLFPPSSEELQANKATLVCLISDFYPGAVTVAWKADSSPVKAGVETTTPSKQSNNKYAASSYLSLTPEQWKSHRSYSCQVTHEGSTVEKTVAPTECS

SEQ ID NO: 30 - DNA, 372 bp, Homo sapiens
  CDS (1)..(372): 30G1-VH variable heavy chain (VH) sequence; 30G1: IgG1, kappa
  V_region (91)..(105): complementarity determining region (CDR) VH-CDR1
  V_region (148)..(198): complementarity determining region (CDR) VH-CDR2
  V_region (295)..(339): complementarity determining region (CDR) VH-CDR3
gaggtgcagctgttggaatcggggggaggcttggttcagccgggggggtccctgagactctcctgtgcagcctctggattcacctttagtacctatgccatgagttgggtccgccaggctccagggaaggggctggagtgggtctcaactataactagcagtggtggtgccacttaccacgcagactccgtgaagggccggctcaccatctccagagacaattccaagaacacgctgtatttggagatgaacagcctgagagtcgaggacacggccgtctattactgtgcgaaagattggggaagaacggtttatgcggtgatcaaggaccttgacatctggggccagggaaccctggtcaccgtctcctca

SEQ ID NO: 31 - protein, 124 aa, Homo sapiens
EVQLLESGGGLVQPGGSLRLSCAASGFTFSTYAMSWVRQAPGKGLEWVSTITSSGGATYHADSVKGRLTISRDNSKNTLYLEMNSLRVEDTAVYYCAKDWGRTVYAVIKDLDIWGQGTLVTVSS

SEQ ID NO: 32 - DNA, 324 bp, Homo sapiens
  CDS (1)..(324): 30G1-VL variable light chain (VL) sequence, kappa type
  V_region (70)..(102): complementarity determining region (CDR) VL-CDR1
  V_region (148)..(168): complementarity determining region (CDR) VL-CDR2
  V_region (265)..(294): complementarity determining region (CDR) VL-CDR3
gaaattgtgatgacacagtctccagccatcctgtctgtgtctccaggggaaagagccaccctctcctgcagggccagtcagagtgttagcaactacttagcctggttccaacaaaagcctggccaggctcccaggctcctcatctatgacacatctaagagggccactggcacccccgccaggttcagtggcagtgggtctgggacagacttcactctcaccatcagcagcctagagcctgaagattttgcagtttatttctgtcagcagcgtagcgactggcctcagtacacttttggccaggggaccaaactggagatcaaa

SEQ ID NO: 33 - protein, 108 aa, Homo sapiens
EIVMTQSPAILSVSPGERATLSCRASQSVSNYLAWFQQKPGQAPRLLIYDTSKRATGTPARFSGSGSGTDFTLTISSLEPEDFAVYFCQQRSDWPQYTFGQGTKLEIK

SEQ ID NO: 34 - DNA, 993 bp, Homo sapiens; identical to SEQ ID NO: 10
  CDS (1)..(990): 30G1-CH constant heavy chain (CH) sequence

SEQ ID NO: 35 - protein, 330 aa, Homo sapiens [sequence omitted]

SEQ ID NO: 36 - DNA, 324 bp, Homo sapiens; identical to SEQ ID NO: 12
  CDS (1)..(321): 30G1-CL constant kappa chain (CL) sequence
  misc_feature (248)..(324): not sequenced but obtained from database

SEQ ID NO: 37 - protein, 107 aa, Homo sapiens [sequence omitted]

SEQ ID NO: 38 - DNA, 378 bp, Homo sapiens
  CDS (1)..(378): 35G11-VH variable heavy chain (VH) sequence; 35G11: IgG4, lambda
  V_region (91)..(105): complementarity determining region (CDR) VH-CDR1
  V_region (148)..(198): complementarity determining region (CDR) VH-CDR2
  V_region (295)..(345): complementarity determining region (CDR) VH-CDR3
caggtgcagctggttcaatctgggtctgagttgaggaggcctggggcctcagtgaacatttcctgcaaggcttctggttacggcttcaatacttatgctatgaattgggtgcgacaggcccctggacaagggcctgagtggatgggatggatcaacaccgacactggggacccaacgtacgcccaggggttcacgggacggtttgccttcttcttggacacgtctgccagcacggcatttctgcagatcactcgcctaacgggtgaggacactgccgtgtatttctgtgcgagaactcggaacaactggaacggcgtttactatcactactccggtttggacgtctggggccaagggaccacggtcaccgtctcctca

SEQ ID NO: 39 - protein, 126 aa, Homo sapiens
QVQLVQSGSELRRPGASVNISCKASGYGFNTYAMNWVRQAPGQGPEWMGWINTDTGDPTYAQGFTGRFAFFLDTSASTAFLQITRLTGEDTAVYFCARTRNNWNGVYYHYSGLDVWGQGTTVTVSS

SEQ ID NO: 40 - DNA, 330 bp, Homo sapiens
  CDS (1)..(330): 35G11-VL variable light chain (VL), lambda type
  V_region (67)..(105): complementarity determining region (CDR) VL-CDR1
  V_region (151)..(171): complementarity determining region (CDR) VL-CDR2
  V_region (268)..(300): complementarity determining region (CDR) VL-CDR3
cagtctgtgctgactcagcctccctctgcgtctgggacccccgggcagacggtcaccatctcctgttctggaagcagccccaacctcggagacaattatgtatactggtaccaccaagtcccaggaacggcccccaaactcctcatttttaggaatactcagcggccctcaggggtcactgaccgattctctggctccaagtatggcacctcagcctccctggccataagtgatctccggtccgacgatgaaggtgatttttactgtgcttcgtgggatgaccgcctgagtcgtctggtgttcggcggagggaccaagctgaccgtccta

SEQ ID NO: 41 - protein, 110 aa, Homo sapiens
QSVLTQPPSASGTPGQTVTISCSGSSPNLGDNYVYWYHQVPGTAPKLLIFRNTQRPSGVTDRFSGSKYGTSASLAISDLRSDDEGDFYCASWDDRLSRLVFGGGTKLTVL

SEQ ID NO: 42 - DNA, 984 bp, Homo sapiens
  CDS (1)..(981): 35G11-CH constant heavy chain (CH) sequence
gcttccaccaagggcccatccgtcttccccctggcgccctgctccaggagcacctccgagagcacagccgccctgggctgcctggtcaaggactacttccccgaaccggtgacggtgtcgtggaactcaggcgccctgaccagcggcgtgcacaccttcccggctgtcctacagtcctcaggactctactccctcagcagcgtggtgaccgtgccctccagcagcttgggcacgaagacctacacctgcaacgtagatcacaagcccagcaacaccaaggtggacaagagagttgagtccaaatatggtcccccatgcccatcatgcccagcacctgagttcctggggggaccatcagtcttcctgttccccccaaaacccaaggacactctcatgatctcccggacccctgaggtcacgtgcgtggtggtggacgtgagccaggaagaccccgaggtccagttcaactggtacgtggatggcgtggaggtgcataatgccaagacaaagccgcgggaggagcagttcaacagcacgtaccgtgtggtcagcgtcctcaccgtcctgcaccaggactggctgaacggcaaggagtacaagtgcaaggtctccaacaaaggcctcccgtcctccatcgagaaaaccatctccaaagccaaagggcagccccgagagccacaggtgtacaccctgcccccatcccaggaggagatgaccaagaaccaggtcagcctgacctgcctggtcaaaggcttctaccccagcgacatcgccgtggagtgggagagcaatgggcagccggagaacaactacaagaccacgcctcccgtgctggactccgacggctccttcttcctctacagcaggctaaccgtggacaagagcaggtggcaggaggggaatgtcttctcatgctccgtgatgcatgaggctctgcacaaccactacacacagaagagcctctccctgtctctgggtaaatga

SEQ ID NO: 43 - protein, 327 aa, Homo sapiens
ASTKGPSVFPLAPCSRSTSESTAALGCLVKDYFPEPVTVSWNSGALTSGVHTFPAVLQSSGLYSLSSVVTVPSSSLGTKTYTCNVDHKPSNTKVDKRVESKYGPPCPSCPAPEFLGGPSVFLFPPKPKDTLMISRTPEVTCVVVDVSQEDPEVQFNWYVDGVEVHNAKTKPREEQFNSTYRVVSVLTVLHQDWLNGKEYKCKVSNKGLPSSIEKTISKAKGQPREPQVYTLPPSQEEMTKNQVSLTCLVKGFYPSDIAVEWESNGQPENNYKTTPPVLDSDGSFFLYSRLTVDKSRWQEGNVFSCSVMHEALHNHYTQKSLSLSLGK

SEQ ID NO: 44 - DNA, 321 bp, Homo sapiens
  CDS (1)..(318): 35G11-CL constant lambda chain (CL) sequence
  variation (211)..(213): tac may be also tat
  misc_feature (250)..(321): not sequenced but obtained from database
ggtcagcccaaggctgccccctcggtcactctgttcccgccctcctctgaggagcttcaagccaacaaggccacactggtgtgtctcataagtgacttctacccgggagccgtgacagtggcctggaaggcagatagcagccccgtcaaggcgggagtggagaccaccacaccctccaaacaaagcaacaacaagtacgcggccagcagctacctgagcctgacgcctgagcagtggaagtcccacagaagctacagctgccaggtcacgcatgaagggagcaccgtggagaagacagtggcccctacagaatgttcatag

SEQ ID NO: 45 - protein, 106 aa, Homo sapiens; identical to SEQ ID NO: 29

SEQ ID NO: 46 - DNA, 354 bp, Homo sapiens
  CDS (1)..(354): 41D11-VH variable heavy chain (VH) sequence; 41D11: IgG1, lambda
  V_region (91)..(111): complementarity determining region (CDR) VH-CDR1
  V_region (154)..(201): complementarity determining region (CDR) VH-CDR2
  V_region (298)..(321): complementarity determining region (CDR) VH-CDR3
caggtgcaactacatgagtcgggcccaggactggtgaagccttcggagaccctgtccgtaacctgcagtctctctggtggctccatcagtagtagtagtcacctgtgggcctggatccgccagcccccagagaagggactggaatatatcgggcgtattcattataggggcagtgtgtcctacaatccgtccctcaagagtcgcgccgccatttccgtcgacacggccaagaaccagttctccctgacgttgagtgctgtgaccgccgcagacacgtctttttattactgtgcgagactggacatgggggcaatagacaagtggggccagggaaccctggtcatcgtctcctca

SEQ ID NO: 47 - protein, 118 aa, Homo sapiens
QVQLHESGPGLVKPSETLSVTCSLSGGSISSSSHLWAWIRQPPEKGLEYIGRIHYRGSVSYNPSLKSRAAISVDTAKNQFSLTLSAVTAADTSFYYCARLDMGAIDKWGQGTLVIVSS

SEQ ID NO: 48 - DNA, 333 bp, Homo sapiens
  CDS (1)..(333): 41D11-VL variable light chain (VL) sequence, lambda type
  V_region (67)..(102): complementarity determining region (CDR) VL-CDR1
  V_region (148)..(180): complementarity determining region (CDR) VL-CDR2
  V_region (277)..(303): complementarity determining region (CDR) VL-CDR3
cagcctgtgctgactcaatcgccctctgcctctgcctccctgggagcctcgatcaaactcacctgcactctgagcagtggacacagcaactacgacatcgcttggcatcaacagcagtcggggaagggccctcgattcttgatgagagttaacaatggtggaagccacaacaagggggacgggatccctgatcgtttctcaggctccagctctggggcagagcgctacctcacaatctccagtctccagtctgaggatgaggctgactattattgtcagacatggggcactggcactcatgtcttcggcactgggactaaggtcaccgtcctg

SEQ ID NO: 49 - protein, 111 aa, Homo sapiens
QPVLTQSPSASASLGASIKLTCTLSSGHSNYDIAWHQQQSGKGPRFLMRVNNGGSHNKGDGIPDRFSGSSSGAERYLTISSLQSEDEADYYCQTWGTGTHVFGTGTKVTVL

SEQ ID NO: 50 - DNA, 993 bp, Homo sapiens
  CDS (1)..(990): 41D11-CH constant heavy chain (CH) sequence
  variation (877)..(879): ttc may be also ctc, thus Phe may be also Leu at position 293 of the amino acid sequence
gcctccaccaagggcccatcggtcttccccctggcaccctcctccaagagcacctctgggggcacagcggccctgggctgcctggtcaaggactacttccccgaaccggtgacggtgtcgtggaactcaggcgccctgaccagcggcgtgcacaccttcccggctgtcctacagtcctcaggactctactccctcagcagcgtggtgaccgtgccctccagcagcttgggcacccagacctacatctgcaacgtgaatcacaagcccagcaacaccaaggtggacaagagagttgagcccaaatcttgtgacaaaactcacacatgcccaccgtgcccagcacctgaactcctggggggaccgtcagtcttcctcttccccccaaaacccaaggacaccctcatgatctcccggacccctgaggtcacatgcgtggtggtggacgtgagccacgaagaccctgaggtcaagttcaactggtacgtggacggcgtggaggtgcataatgccaagacaaagccgcgggaggagcagtacaacagcacgtaccgtgtggtcagcgtcctcaccgtcctgcaccaggactggctgaatggcaaggagtacaagtgcaaggtctccaacaaagccctcccagcccccatcgagaaaaccatctccaaagccaaagggcagccccgagaaccacaggtgtacaccctgcccccatcccgggaggagatgaccaagaaccaggtcagcctgacctgcctggtcaaaggcttctatcccagcgacatcgccgtggagtgggagagcaatgggcagccggagaacaactacaagaccacgcctcccgtgctggactccgacggctccttcttcctctatagcaagttcaccgtggacaagagcaggtggcagcaggggaacgtcttctcatgctccgtgatgcatgaggctctgcacaaccactacacgcagaagagcctctccctgtccccgggtaaatga

SEQ ID NO: 51 - protein, 330 aa, Homo sapiens
ASTKGPSVFPLAPSSKSTSGGTAALGCLVKDYFPEPVTVSWNSGALTSGVHTFPAVLQSSGLYSLSSVVTVPSSSLGTQTYICNVNHKPSNTKVDKRVEPKSCDKTHTCPPCPAPELLGGPSVFLFPPKPKDTLMISRTPEVTCVVVDVSHEDPEVKFNWYVDGVEVHNAKTKPREEQYNSTYRVVSVLTVLHQDWLNGKEYKCKVSNKALPAPIEKTISKAKGQPREPQVYTLPPSREEMTKNQVSLTCLVKGFYPSDIAVEWESNGQPENNYKTTPPVLDSDGSFFLYSKFTVDKSRWQQGNVFSCSVMHEALHNHYTQKSLSLSPGK

SEQ ID NO: 52 - DNA, 321 bp, Homo sapiens
  CDS (1)..(318): 41D11-CL constant lambda chain (CL) sequence
  misc_feature (250)..(321): not sequenced but obtained from database
ggtcagcccaaggccaaccccactgtcactctgttcccgccctcctctgaggagctccaagccaacaaggccacactagtgtgtctgatcagtgacttctacccgggagctgtgacagtggcctggaaggcagatggcagccccgtcaaggcgggagtggagaccaccaaaccctccaaacagagcaacaacaagtacgcggccagcagctacctgagcctgacgcccgagcagtggaagtcccacagaagctacagctgccaggtcacgcatgaagggagcaccgtggagaagacagtggcccctacagaatgttcatag

SEQ ID NO: 53 - protein, 106 aa, Homo sapiens
GQPKANPTVTLFPPSSEELQANKATLVCLISDFYPGAVTVAWKADGSPVKAGVETTKPSKQSNNKYAASSYLSLTPEQWKSHRSYSCQVTHEGSTVEKTVAPTECS

SEQ ID NO: 54 - DNA, 357 bp, Homo sapiens
  CDS (1)..(357): 51G4-VH-variable heavy chain (VH) sequence; 51G4: IgG2, lambda
  misc_feature (1)..(18): not sequenced but derived from primer used for molecular cloning
  V_region (91)..(105): complementarity determining region (CDR) VH-CDR1
  V_region (148)..(198): complementarity determining region (CDR) VH-CDR2
  V_region (295)..(324): complementarity determining region (CDR) VH-CDR3
  misc_feature (340)..(357): not sequenced but derived from primer used for molecular cloning
gaggtgcagctggtgcagtctggggctgaggtgaagaagcctggggcctcagtgaaggtttcatgtaaaacttctggatacaaattcgctctctatgatattcattgggtgcgccaggcccccggacaagggcttgagtggatgggctggatcaacgctgccaatggtgacacagaatattcacagaagtttgagggcagagtcaccattaccagggacacatcggcgactacagtctacatggagttgaacagtctgacatatggcgacacggccgtgtactactgtgcgagagaggaaggtctctacaactggttcgacccctggggccagggaaccctggtcaccgtctcctca

SEQ ID NO: 55 - protein, 119 aa, Homo sapiens
EVQLVQSGAEVKKPGASVKVSCKTSGYKFALYDIHWVRQAPGQGLEWMGWINAANGDTEYSQKFEGRVTITRDTSATTVYMELNSLTYGDTAVYYCAREEGLYNWFDPWGQGTLVTVSS

SEQ ID NO: 56 - DNA, 327 bp, Homo sapiens
  CDS (1)..(327): 51G4-variable light chain (VL) sequence, lambda type
  misc_feature (1)..(18): not sequenced but derived from primer used for molecular cloning
  V_region (67)..(99): complementarity determining region (CDR) VL-CDR1
  V_region (145)..(165): complementarity determining region (CDR) VL-CDR2
  V_region (262)..(297): complementarity determining region (CDR) VL-CDR3
tcctatgagctgacacaggaccctgctgtgtctgtggccttgggacagacagtcaggatcacatgccaaggagacagcctcagaatctattatgcaaactggtaccagcagaagccaggacaggcccctgttcttgtcatctatggtaaaagcaaccggccctcagggatcccagaccgattctctgcctccagctcaggaaacacagcttccttgaccatcactggggctcaggcggaagatgaggctgactattactgtaactcccgggacagcagtgataagcatcccgtgcctttcggcggggggaccaagctgaccgtccta

SEQ ID NO: 57 - protein, 109 aa, Homo sapiens
SYELTQDPAVSVALGQTVRITCQGDSLRIYYANWYQQKPGQAPVLVIYGKSNRPSGIPDRFSASSSGNTASLTITGAQAEDEADYYCNSRDSSDKHPVPFGGGTKLTVL

SEQ ID NO: 58 - DNA, 981 bp, Homo sapiens
  CDS (1)..(978): 51G4-CH constant heavy chain (CH) sequence
  misc_feature (1)..(47): not sequenced but obtained from database
gcctccaccaagggcccatcggtcttccccctggcgccctgctccaggagcacctccgagagcacagcggccctgggctgcctggtcaaggactacttccccgaaccggtgacggtgtcgtggaactcaggtgctctgaccagcggcgtgcacaccttcccagctgtcctacagtcctcaggactctactccctcagcagcgtggtgaccgtgccctccagcaacttcggcacccagacctacacctgcaacgtagatcacaagcccagcaacaccaaggtggacaagacagttgagcgcaaatgttgtgtcgagtgcccaccgtgcccagcaccacctgtggcaggaccgtcagtcttcctcttccccccaaaacccaaggacaccctcatgatctcccggacccctgaggtcacgtgcgtggtggtggacgtgagccacgaagaccccgaggtccagttcaactggtacgtggacggcgtggaggtgcataatgccaagacaaagccacgggaggagcagttcaacagcacgttccgtgtggtcagcgtcctcaccgttgtgcaccaggactggctgaacggcaaggagtacaagtgcaaggtctccaacaaaggcctcccagcccccatcgagaaaaccatctccaaaaccaaagggcagccccgagaaccacaggtgtacaccctgcccccatcccgggaggagatgaccaagaaccaggtcagcctgacctgcctggtcaaaggcttctaccccagcgacatcgccgtggagtgggagagcaatgggcagccggagaacaactacaagaccacacctcccatgctggactccgacggctccttcttcctctacagcaagctcaccgtggacaagagcaggtggcagcaggggaacgtcttctcatgctccgtgatgcatgaggctctgcacaaccactacacgcagaagagcctctccctgtctccgggtaaatga

SEQ ID NO: 59 - protein, 326 aa, Homo sapiens
ASTKGPSVFPLAPCSRSTSESTAALGCLVKDYFPEPVTVSWNSGALTSGVHTFPAVLQSSGLYSLSSVVTVPSSNFGTQTYTCNVDHKPSNTKVDKTVERKCCVECPPCPAPPVAGPSVFLFPPKPKDTLMISRTPEVTCVVVDVSHEDPEVQFNWYVDGVEVHNAKTKPREEQFNSTFRVVSVLTVVHQDWLNGKEYKCKVSNKGLPAPIEKTISKTKGQPREPQVYTLPPSREEMTKNQVSLTCLVKGFYPSDIAVEWESNGQPENNYKTTPPMLDSDGSFFLYSKLTVDKSRWQQGNVFSCSVMHEALHNHYTQKSLSLSPGK

SEQ ID NO: 60 - DNA, 321 bp, Homo sapiens
  CDS (1)..(318): 51G4-CL constant lambda chain (CL) sequence
  misc_feature (27)..(321): not sequenced but obtained from lambda constant chain of 24D3 from the same patient
agtcagcccaaggctgccccctcggtcactctgttcccgccctcctctgaggagcttcaagccaacaaggccacactggtgtgtctcataagtgacttctacccgggagccgtgacagtggcctggaaggcagatagcagccccgtcaaggcgggagtggagaccaccacaccctccaaacaaagcaacaacaagtacgcggccagcagctatctgagcctgacgcctgagcagtggaagtcccacagaagctacagctgccaggtcacgcatgaagggagcaccgtggagaagacagtggcccctacagaatgttcatag

SEQ ID NO: 61 - protein, 106 aa, Homo sapiens
SQPKAAPSVTLFPPSSEELQANKATLVCLISDFYPGAVTVAWKADSSPVKAGVETTTPSKQSNNKYAASSYLSLTPEQWKSHRSYSCQVTHEGSTVEKTVAPTECS

SEQ ID NO: 62 - DNA, 34 bp, Artificial Sequence
  Forward Oligonucleotide/Primer F1 for amplification of a fragment encoding aa 34-76 of IL-22
tttgggatcctcgcgcccatcagctcccactgca

SEQ ID NO: 63 - DNA, 35 bp, Artificial Sequence
  Reverse Oligonucleotide/Primer R1 for amplification of a fragment encoding aa 34-76 of IL-22
tttgcggccgctcacccaatgagacgaacgtctgt

SEQ ID NO: 64 - DNA, 34 bp, Artificial Sequence
  Forward oligonucleotide/primer F2 for amplification of a fragment encoding aa 74-114 of IL-22
tttgggatcctcctcattggggagaaactgttcc

SEQ ID NO: 65 - DNA, 35 bp, Artificial Sequence
  Reverse oligonucleotide/primer R2 for amplification of a fragment encoding aa 74-114 of IL-22
tttgcggccgctcaataaggctggaacctatcaga

SEQ ID NO: 66 - DNA, 32 bp, Artificial Sequence
  Forward oligonucleotide/primer F3 for amplification of a fragment encoding aa 113-179 of IL-22
tttgggatcctcccttatatgcaggaggtggt

SEQ ID NO: 67 - DNA, 33 bp, Artificial Sequence
  Reverse oligonucleotide/primer R3 for amplification of a fragment encoding aa 113-179 of IL-22
tttgcggccgctcaaatgcaggcatttctcaga

SEQ ID NO: 68 - DNA, 34 bp, Artificial Sequence; identical to SEQ ID NO: 62
  Forward oligonucleotide/primer 34-114-F1 for amplification of a fragment encoding aa 34-114 of IL-22

SEQ ID NO: 69 - DNA, 35 bp, Artificial Sequence; identical to SEQ ID NO: 65
  Reverse oligonucleotide/primer 34-114-R2 for amplification of a fragment encoding aa 34-114 of IL-22

SEQ ID NO: 70 - DNA, 34 bp, Artificial Sequence; identical to SEQ ID NO: 64
  Forward oligonucleotide/primer 74-179-F2 for amplification of a fragment encoding aa 74-179 of IL-22

SEQ ID NO: 71 - DNA, 33 bp, Artificial Sequence; identical to SEQ ID NO: 67
  Reverse oligonucleotide/primer 74-179-R3 for amplification of a fragment encoding aa 74-179 of IL-22

SEQ ID NO: 72 - DNA, 34 bp, Artificial Sequence
  Forward oligonucleotide/primer F1 for amplification of a fragment encoding aa 24-69 of IFN-alpha2a
tttgggatcctctgtgatctgcctcaaacccaca

SEQ ID NO: 73 - DNA, 35 bp, Artificial Sequence
  Reverse oligonucleotide/primer R1 for amplification of a fragment encoding aa 24-69 of IFN-alpha2a
tttgcggccgctcactggttgccaaactcctcctg

SEQ ID NO: 74 - DNA, 33 bp, Artificial Sequence
  Forward oligonucleotide/primer F2 for amplification of a fragment encoding aa 67-124 of IFN-alpha2a
tttgggatcctcggcaaccagttccaaaaggct

SEQ ID NO: 75 - DNA, 35 bp, Artificial Sequence
  Reverse oligonucleotide/primer R2 for amplification of a fragment encoding aa 67-124 of IFN-alpha2a
tttgcggccgctcactgtatcacacaggcttccag

SEQ ID NO: 76 - DNA, 33 bp, Artificial Sequence
  Forward oligonucleotide/primer F3 for amplification of a fragment encoding aa 123-188 of IFN-alpha2a
tttgggatcctcatacagggggtgggggtgaca

SEQ ID NO: 77 - DNA, 33 bp, Artificial Sequence
  Reverse oligonucleotide/primer R3 for amplification of a fragment encoding aa 123-188 of IFN-alpha2a
tttgcggccgcttacttcttaaactttcttgca

SEQ ID NO: 78 - DNA, 34 bp, Artificial Sequence; identical to SEQ ID NO: 72
  Forward oligonucleotide/primer 24-124-F1 for amplification of a fragment encoding aa 24-124 of IFN-alpha2a

SEQ ID NO: 79 - DNA, 35 bp, Artificial Sequence; identical to SEQ ID NO: 75
  Reverse oligonucleotide/primer 24-124-R2 for amplification of a fragment encoding aa 24-124 of IFN-alpha2a

SEQ ID NO: 80 - DNA, 33 bp, Artificial Sequence; identical to SEQ ID NO: 74
  Forward oligonucleotide/primer 67-188-F2 for amplification of a fragment encoding aa 67-188 of IFN-alpha2a

SEQ ID NO: 81 - DNA, 33 bp, Artificial Sequence; identical to SEQ ID NO: 77
  Forward oligonucleotide/primer 67-188-F3 for amplification of a fragment encoding aa 67-188 of IFN-alpha2a